European Patent Specification EP 2 844 062 B1, published April 8, 2026. Title: Methods and Compositions for Producing Plants with Elevated Brix. Applicant: Bachlava, Eleni King, Joseph  J. Krishnamurthy, Subash Mills, Jeffrey  M. Wentzell, Adam  M. Application Unknown. The sequence listing filed with the application follows.

SEQUENCE LISTING (110 sequences)

SEQ ID NO: 1 - DNA, 121 bp, Cucumis melo
cgagtcaaggcaagctggaggacgcactgtatcgcagtcatgctcgacaggacatgttgcmtgtggccgcatgatcgctccgacaccttttactattttctttcatcgtattttagtttct

SEQ ID NO: 2 - DNA, 121 bp, Cucumis melo
tgttggatttaagaagactttaaatgctatcatctcacagctacctaagcacagacaaacstttctgttctcagcaactcaaacgaagtctgttcaggatcttgccagactcagtttgaaa

SEQ ID NO: 3 - DNA, 121 bp, Cucumis melo
ttggtcgttttggtgtgtcggtattcaagttgattagtttgtttgtagcttttaagttcgyaactgtttggtaggagctctgatagaattttacttgctgtttatatacttctgtttccct

SEQ ID NO: 4 - DNA, 121 bp, Cucumis melo
ctctcacagtggcgcagcctttcgcctcctcgaatctgtcacatttttagggcggacatgrtaggtgttatctttggctgttgggaaatataaagtgaaataaaacatttgtgtgtggtga

SEQ ID NO: 5 - DNA, 121 bp, Cucumis melo
ccaaataagcctggaagatgactcagtatattcttcaccattttaactacgaaatcttttsgattcctggacattttcatttcgcttgcttttgattcttcctcctggataacattttctt

SEQ ID NO: 6 - DNA, 121 bp, Cucumis melo
  misc_feature (118)..(118): n is a, c, g, or t
cacccatgctgatgcactacgcctggcactagaaatgagtccatacgagagagaaaatccrtccaagactgcaggaagagggacaaccccaggtcagaagaggaaggctgagttgcancct

SEQ ID NO: 7 - DNA, 121 bp, Cucumis melo
tgaaaagaagaagattccatcgaatattccatctgttcccattgatgaagttttgtttcayctcgaagaaagcatgcaaagataaaaatatgtagtgcaaaggcatattgcagatgaggtg

SEQ ID NO: 8 - DNA, 121 bp, Cucumis melo
  misc_feature (100)..(100): n is a, c, g, or t
acttgattcttagttcctcttacaacatcaactcttcattcaacgtgttatgtatatacayagttctaacccttctctattttcactctcttattgaaanttttttctttggctttgttga

SEQ ID NO: 9 - DNA, 121 bp, Cucumis melo
  misc_feature (4)..(4): n is a, c, g, or t
tggnaatccttataactaaaagcaaaagaaagacctttgtcttgcaattctcttaagtcaycaacctttggttggttccatgctaaattttgtatggctttgttttcttcagcatcccctc

SEQ ID NO: 10 - DNA, 121 bp, Cucumis melo
  misc_feature (7)..(32): n is a, c, g, or t
gacgggnnnnnnnnnnnnnnnnnnnnnnnnnnatcattgatcgagggtattgcaatttgtyagttactgtggaactatggaatccttatcgtttgtgaagtttggttgagtttgtatgctt

SEQ ID NO: 11 - DNA, 103 bp, Cucumis melo
atctcttctctctctcctcttgctctctctttcaccctcttatgttcttgctgattcccaytttgaaggatttgaaccagaactcgacgacctcgaagatgac

SEQ ID NO: 12 - DNA, 99 bp, Cucumis melo
atcggaatacacaactcaagattctctctccctcctcgygcatgaaccaagatgaaaccatctgtattcttttcttctcttcatcttctctccaccttc

SEQ ID NO: 13 - DNA, 121 bp, Cucumis melo
aaaaaagagattgaagtgcacgattgtatacagagatgcacttacatcaatattgagtgargttaaccattgccttggtaggtgccgggttagatgttcgtccacaatggcaaggcgaggg

SEQ ID NO: 14 - DNA, 107 bp, Cucumis melo
  misc_feature (93)..(96): n is a, c, g, or t
  misc_feature (98)..(101): n is a, c, g, or t
  misc_feature (103)..(104): n is a, c, g, or t
ccacaaccctttacccccatgaaaaattttcctactctccaatcacwtttgcaatagcatcaagcaaaagacaaataacaattacatcccaannnncnnnnannacc

SEQ ID NO: 15 - DNA, 121 bp, Cucumis melo
aaacctattcgccttcttcttcctcaagaaaatcctaaagaaaccctaaccctaaaaaccsttgcaccgctgctgctgtcactcgcctccgtcctacatcgctatttttctttcgtaagcc

SEQ ID NO: 16 - DNA, 121 bp, Cucumis melo
  misc_feature (105)..(105): n is a, c, g, or t
  misc_feature (121)..(121): n is a, c, g, or t
tctaaaaagtggcaaacatatgtccttgtcaaacagcaccgaagtgctccaacaaagaaawttggctatgttcaagtacttcttctattcgcccccaaataactntgaacgacaatgaccn

SEQ ID NO: 17 - DNA, 121 bp, Cucumis melo
gaagggatcaacatcagcccagttttcaacattgcagacctcaaaaggtacaatgcgcctratggattccagcttacaatagcagacgcaacttgaggacaagtttgatgctcaggggatg

SEQ ID NO: 18 - DNA, 121 bp, Cucumis melo
ttgagattattaggagaaactagatctactgtctttgaaaattgtctcatttttccattgygggttttggccagtctaataacttttagttgatcatttctctttactctgtgcttcattg

SEQ ID NO: 19 - DNA, 121 bp, Cucumis melo
ttaagtacctaatagattagtacctaagaaggtgtgatactatttttgggtctttggtgcwagtgagaatgcacaggagatggcttgttgttggtgctgccacggtgaaattgcaaataga

SEQ ID NO: 20 - DNA, 121 bp, Cucumis melo
gcatctgttttcatagaatctgagcagaagcctctctgttgtctgcatttggattctcagyaactttgttctcaactcttctgaaaacaagtttttgctgagggagttggccgttagagac

SEQ ID NO: 21 - DNA, 121 bp, Cucumis melo
ttatagcaagattaaccaaactacacgatgaaccatctgttctaagtacttgaaccctctytatcctaagatctttctcagggcctaaatcactcactaaaatattgtctatcctcttcac

SEQ ID NO: 22 - DNA, 121 bp, Cucumis melo
acgcatgcgctcatatatgtaatccttatacgtggtggatggtcagcctttggtgagaacrcctatatgtttaaaaccatcttgcatatggatgaacatcttgtttctatgagttattgtt

SEQ ID NO: 23 - DNA, 121 bp, Cucumis melo
  misc_feature (113)..(113): n is a, c, g, or t
acatggagggttgaatgtgaattcatcgtcctcttcaccaatagaactatattctgatccwggaagtcctgaaaataatcattcttctatctccagtcctccaaaggttgggnaatgtcca

SEQ ID NO: 24 - DNA, 121 bp, Cucumis melo
  misc_feature (10)..(10): n is a, c, g, or t
  misc_feature (94)..(94): n is a, c, g, or t
actagatatntagtaatatttcagttaaggggtataagggtaattggataacataggaagytactagtagttattgtgttagtgtgattactanggtgattacaacctgttataaatagag

SEQ ID NO: 25 - DNA, 121 bp, Cucumis melo
tgtggccatatatctcgggtcctgcttgttccagcctaatcgaaccaagggagtgtcaggytcggagctctcgtagataatagtagagtgctccttatcgcgcaaatcgaagacccggaca

SEQ ID NO: 26 - DNA, 121 bp, Cucumis melo
ttcactcgtcggaggaacactagaggtatgatcaaggaatttctcctcaacccatctaatrggaagaagggtcattttctattatgactcattgaggtgtgggcgatcttctgaaccttgt

SEQ ID NO: 27 - DNA, 121 bp, Cucumis melo
accttcgggaagaggcagatgagagtttcatttaatgatgcattgatagaaccataagagyagaagtcaataatcatgttcttaatgtcttgcttgagagaaggctagaaaaattttaaaa

SEQ ID NO: 28 - DNA, 121 bp, Cucumis melo
  misc_feature (106)..(106): n is a, c, g, or t
gttgtggctttggaagtgtgctttgacggtgaaggaaggcttgtctcaccagctaccttaraggttgtttccttcctcttttagagcgggtcatcactgccttctncaaggcttcttttct

SEQ ID NO: 29 - DNA, 101 bp, Cucumis melo
ctgatacaaaaaagcttgaatgaagtaaaatggcaatataygttattcaacttgaaatcaagagctaaatgtagatgtcgagggagatatcaatgacttga

SEQ ID NO: 30 - DNA, 121 bp, Cucumis melo
  misc_feature (84)..(84): n is a, c, g, or t
  misc_feature (114)..(114): n is a, c, g, or t
tagaaccaggatcggtatcaaataggctcgacgggattgaccttctttagtagacctataygacctacaggtgttcaggttggnagtgggctgtggcactaaaatcgactgagnaatttgt

SEQ ID NO: 31 - DNA, 121 bp, Cucumis melo
tgagttcgtcaatttgcatttgatgattgcttgcgttgtcaactttaagctctaactcttrcaactgttttttactctacaaatgtgtttcttataagttgctttggcattgaattacatc

SEQ ID NO: 32 - DNA, 121 bp, Cucumis melo
  misc_feature (96)..(96): n is a, c, g, or t
tttattcttttttgctcttcacaagcaagattaggaaatctattgtaggatgtaggactcraaggtaaatatataacacaataaatctcaggtagnaaaatttgccgaatattggaagaag

SEQ ID NO: 33 - DNA, 121 bp, Cucumis melo
  misc_feature (23)..(23): n is a, c, g, or t
ttgcttttcgacctgaaaacttngatatgatcactaccaagaacaccaaaccggaaatcayccacagagcaataatccacgacctcaaagaactaaagatcccatcctcttttgcctccac

SEQ ID NO: 34 - DNA, 121 bp, Cucumis melo
ctttcttttgccttctcttagtactggagacgagaaagtaatcagtggtcttgcatgcttrttctcagaagttgggcaagcagtatgttgctgtggactcctgtttgtgttataattatta

SEQ ID NO: 35 - DNA, 121 bp, Cucumis melo
ctgcaggcttccacatcttcaatgtaaaaatgccttcctctgtccaatgcaatagtgcaaytggcttacttttcagctaactacctccacttttgttttgaagctcgccggaggagactgg

SEQ ID NO: 36 - DNA, 98 bp, Cucumis melo
  misc_feature (6)..(6): n is a, c, g, or t
acatantcccccttctctcgcacaaacattaaatgcacgtcaaccaacatcacgccacccrtcgactctccctccaccagctttgctggcagcaggac

SEQ ID NO: 37 - DNA, 121 bp, Cucumis melo
ttgtaaggtccaaagagttttggagataatttttcattccttttctttctcaaggatgtcwgatggtacaacctaattgcttttttctcattctcctgttcaatcactttcatctatgttt

SEQ ID NO: 38 - DNA, 121 bp, Cucumis melo
  misc_feature (31)..(31): n is a, c, g, or t
  misc_feature (87)..(87): n is a, c, g, or t
ttgacagcagtatttccaacgtcaatgagtnggtctgacggctaaatggtacttcggcttrgctgaacgtctcttttcttctctccngtgctgatgagtgttcatgattgatttgcagaag

SEQ ID NO: 39 - DNA, 121 bp, Cucumis melo
gcttcagtttctccttgaatataccaaacatgctgtgggccttcatacttgattatatcgwagtgcaagatttcatccttactttattgctttttgaactgtatgctttctgtggggatat

SEQ ID NO: 40 - DNA, 121 bp, Cucumis melo
  misc_feature (107)..(107): n is a, c, g, or t
  misc_feature (116)..(116): n is a, c, g, or t
  misc_feature (118)..(118): n is a, c, g, or t
agatcagagagttttgagcagtaaagccagcttccataattatatgcttcaactaacaatkagagccacaaattcacatctacaattacatttaaccttcatttgtnaaaaaaaantngca

SEQ ID NO: 41 - DNA, 121 bp, Cucumis melo
ttctattctcctttcttagcactgcagagaaatccggcaccgattgcgccaccgtagcggwccttttccttacagtctccgaacccagaaatttaatttgcttcttgggcgggggggtgga

SEQ ID NO: 42 - DNA, 121 bp, Cucumis melo
  misc_feature (111)..(111): n is a, c, g, or t
acttttgctgaaactcatagcataattattatttgtatacctatatatcccttcattggawgctacttagctttattcttttattggtttctttgagattaattgctagcntcagttctca

SEQ ID NO: 43 - DNA, 121 bp, Cucumis melo
taggggaaggctctaacaaatgaagaggttggagaatcacaaactagaggaccacgaccartggacaagttgatcctaggtagaaataataaaaagtcaatgcattcgaacttgagaaggt

SEQ ID NO: 44 - DNA, 121 bp, Cucumis melo
  misc_feature (17)..(17): n is a, c, g, or t
  misc_feature (20)..(20): n is a, c, g, or t
aagttcttttggattcnttnggttttattaaatggggaatgccaatcaatgctttgcaatsgaaaggaggggttgcattctgataggactcctatctttgatatgaaattcttctttattt

SEQ ID NO: 45 - DNA, 121 bp, Cucumis melo
  misc_feature (26)..(26): n is a, c, g, or t
cgaagctgtggaaggtttctgtgccnaaaaagaaaggttgggtcttaaagctggatttggwaaaggcctttgatcatgtggattgggtgttccttgaaaagttgcttctttgtaaaatgtt

SEQ ID NO: 46 - DNA, 121 bp, Cucumis melo
ataagaggaccctacaagtacttgaaaatttctagatttcttttgaaattctaatccactrggaaacttcatttttgtgctatcttagattcttattacttgcttcctttgattcttatac

SEQ ID NO: 47 - DNA, 121 bp, Cucumis melo
  misc_feature (10)..(11): n is a, c, g, or t
  misc_feature (29)..(29): n is a, c, g, or t
  misc_feature (120)..(120): n is a, c, g, or t
tgtataaatnncaaagtactattgcactnccaatacaagatagaggaaatttctcccatawttgcaaactacgatttcttacttggcatcagagcattgaaatggccaacatcgtctccnt

SEQ ID NO: 48 - DNA, 121 bp, Cucumis melo
tttcaaggagttgggactcacatttgcatctgatggaatttgcatataataacagttatcrtgctaccattgacatgacaccattttaagctttgtgcgataagtgttgcagattctctat

SEQ ID NO: 49 - DNA, 121 bp, Cucumis melo
tcatgaacgtgaacttcgaatggcagaccccgtaggccctcatttcatccattcattttcrttcccattctttgtctgattgtgttggctgtcacggcgccatagattttgtttgtggttc

SEQ ID NO: 50 - DNA, 121 bp, Cucumis melo
  misc_feature (102)..(102): n is a, c, g, or t
tccgattggatggtggaggtggagggcgctaaactgtattatcaagggactttttgcttaytttcccattggacactcccttaatatcaacggtccattccncacgcataatttcgatgat

SEQ ID NO: 51 - DNA, 121 bp, Cucumis melo
ttcattctgagaagcattgacttaaaattcatgtgctgtgcacagacatactgctactatkctccttgtatcagaagccaaacacataggctgggacttgtcaaagaatctacctaactgc

SEQ ID NO: 52 - DNA, 121 bp, Cucumis melo
gaattccttatcaaatattgcaatttcagaccaattactctcacaagcttgacttacaagkttgttgccaaggtgctgtccgaaagactcaaaggcaattccttgcatcattgccccctca

SEQ ID NO: 53 - DNA, 121 bp, Cucumis melo
gaatactcattaaattccttgttcaaagaacaccaagctgctgcatttctttttgcagtgyccgaagtttcagaccagccccttgacttgttatgaaagattcgttgattacgttcaaacc

SEQ ID NO: 54 - DNA, 121 bp, Cucumis melo
agcgcttgaaaaactgagaagattgggaactagaatctgacctatttatattaatcggttsaaggagttgagagcaatgggcttccaacaagtttgggttgttcttggtaagttgagacct

SEQ ID NO: 55 - DNA, 121 bp, Cucumis melo
  misc_feature (5)..(5): n is a, c, g, or t
ttttngtccccttgtattcatttccaagagattgtcttcattggagggcagccaaccaatyagatagataatgaacttcaattaagccaaaagaactctgcaatccttgacaatggaagtt

SEQ ID NO: 56 - DNA, 121 bp, Cucumis melo
aaagtaagttgaattagttacatttgggagacaaaaacacaagctcttttcacatatccckggcagccaaaagaagaaagaatctgaatacagagttagttaatgactccggggtgcccac

SEQ ID NO: 57 - DNA, 99 bp, Cucumis melo
ttgaaggtttggaagaaccatcaccagcaaagaaataaaaaatctcctcatgtaagtcaayccaatcatctcaaagaagacaaaataaaactttgcaaa

SEQ ID NO: 58 - DNA, 103 bp, Cucumis melo
gagtattttcataattttgttgtgcatgattgatgtggcattaaggttttattaggaggcyatcttacttaaatcgtcaataacatttagatgtgattaatct

SEQ ID NO: 59 - DNA, 121 bp, Cucumis melo
gaatgaaacattagtcatgcagtggttatccaagaactgccatactgttttgaacaatctwccaacatcaattgaagaagacgatcagcttctgtgcaatatcgccaaagtccaagatttg

SEQ ID NO: 60 - DNA, 121 bp, Cucumis melo
gaaagggtgctagcagttcttcatcttcatatgagcaagagatgcattccagagaggtttkcgaactaagacctaaccttgaaaatgctcaataattaattgacgaacaatgaagaacgtc

SEQ ID NO: 61 - DNA, 121 bp, Cucumis melo
aagatgaagaaaataacaataaggaagatataaaaaatgatcattactgaaagtgagttgragccaaatcaggcgaaaaatcttaatcttaaaaatttaaaaaccactacaaacttggaaa

SEQ ID NO: 62 - DNA, 121 bp, Cucumis melo
ttgatcgtggaatgttcacacatgaagatattaatggcgcagaccttttggttcaataatyggttgcattggaatttgtatagtgaaacttgtgtggtttgaaggttgcaaataatgagat

SEQ ID NO: 63 - DNA, 121 bp, Cucumis melo
  misc_feature (26)..(26): n is a, c, g, or t
ttgctcttctttttggacagaatgangggagtatgagttggagtacctctcaggaatttcmcctttgaattaggcattgagaagctagagtattcaaagtgttgaagatgagaggattcag

SEQ ID NO: 64 - DNA, 121 bp, Cucumis melo
  misc_feature (4)..(4): n is a, c, g, or t
gatngtttcttcatcaataaggtgtgggattaaatctttgacaacacaagaatcacccgasaagcatgcactttctttgatcatttcccagagtttggagaaaggtggaaacattgtcctt

SEQ ID NO: 65 - DNA, 121 bp, Cucumis melo
atgggccaaaaatcacaacttagcacccacccatctttaccaatgaatttcgacacttccrgtcttccttgatctagctccccaaagttatgaaagaaaccatcttctggacctcttataa

SEQ ID NO: 66 - DNA, 121 bp, Cucumis melo
  misc_feature (15)..(15): n is a, c, g, or t
cacaatttacctcancacatccttttttatttttcacgacacaacgtcttcattggtagtrtcattaaaacccatttttctagtagtgatttctaattttaggttacatgcaagagaaaag

SEQ ID NO: 67 - DNA, 121 bp, Cucumis melo
ttcaataccagtgtcttctctcgatgccggtggcactgttccaggccaacctgagctcctycctcccaactccctcgacgactcgttccggagtgcatccttctccaaagccatagatcat

SEQ ID NO: 68 - DNA, 121 bp, Cucumis melo
aaataagaataatgatgcatattatttaccgcctccaaggaaaaaaaagcacatttggggytgtttggcccaacttcaaatgggtgctcctgtgtctgggacttcaattacaatatatggt

SEQ ID NO: 69 - DNA, 121 bp, Cucumis melo
aaaaggaatggagcttgcaaaggttcttagagatgcgcaggaatgcaatagttcagatacraagcatcaagaatgcaagaagccggaacagcagaatggttctacaactgctaatgcgact

SEQ ID NO: 70 - DNA, 121 bp, Cucumis melo
aggcaatctcgaggattcttgtcgtctgagaggaatgccttctccaccactaaatccatcytcctcggcatgcttagagagccgtattgataagtttgccgctggacctgtatcaatttgc

SEQ ID NO: 71 - DNA, 121 bp, Cucumis melo
tttactttcaaacggtggaagaaggtgttgaacctgaccatttcacttttcctcgtgtgcwcaaggcctgtggtggcattgggtcgattcaaactggagaggcggtgcatcggcatgttgt

SEQ ID NO: 72 - DNA, 121 bp, Cucumis melo
attttggtccataaccaaagtctcaggagagctgtgcactaaaatgctagataatttacgkagtgctcaggaatgctataatgcaaaaggaacatataagatccatagtagaaaccatgtt

SEQ ID NO: 73 - DNA, 121 bp, Cucumis melo
gtttaaccaattataagtcaattgaataagatcagcatcatgacaaataaaataagctcaytcagaaatcaacataggcctactgatcaagaagcaacctctaagcacatattttcatttt

SEQ ID NO: 74 - DNA, 121 bp, Cucumis melo
  misc_feature (108)..(108): n is a, c, g, or t
attgggtccattgtttttgtttctaagataatcttccaaacttcaagattagcaattccartccttgacctccatttcggtccttgagaacgtgatggaaaaaaaatnatacaattcaaaa

SEQ ID NO: 75 - DNA, 121 bp, Cucumis melo
taaaaggtcaatcagaaactccatgaacctctcgcaatacaaaatacaagcattgtctccmtctatcaacccattggcatcaacagattgactgtttgcatcatctgaattattctgaggg

SEQ ID NO: 76 - DNA, 121 bp, Cucumis melo
ggccaaacacgtagagatttttgtacttctgacctagaatcactagacacaatgtcacgarcatctgaaattgaggaagaattgctaatctcaagaaatgattgggtatctgcggaacagg

SEQ ID NO: 77 - DNA, 121 bp, Cucumis melo
ctcttactaaaaaagagatcagtgtatgtcttccttcttcgtttttctatcactttaaggytgattctattcggttcaaagctatgtttgcactctttcctacctttttcgttaatatttg

SEQ ID NO: 78 - DNA, 121 bp, Cucumis melo
agtggcacatgttttggttcggactttgttatgtgaaacaaataaaatgttcattaattgmgtttgcattgcattatttacaagtattactcaatgtattatatgaaaccttaggggaatt

SEQ ID NO: 79 - DNA, 121 bp, Cucumis melo
aaggaattctatgtttgtagtttgaatgtttggtgaagagagtgcaaaaaggtcctccaasgtaagatttaatacccactgtaagcagattttttgtagacgataatatataaagcaatca

SEQ ID NO: 80 - DNA, 95 bp, Cucumis melo
  misc_feature (87)..(92): n is a, c, g, or t
aaaagggggaaaaacctcaaagcttaccttcactrcctcgtccagctcaaagcccagcagcagcaacgcctgtaataatgaacagtnnnnnnttt

SEQ ID NO: 81 - DNA, 121 bp, Cucumis melo
atcctaagctaccaactttaattgctttgagaaatggtaacttttttctccattcatagcytgaaatgaatttgtctgagttgctcaattctataaatatggtatggtcgtccattttatc

SEQ ID NO: 82 - DNA, 121 bp, Cucumis melo
catttttgatgaatatgtatatgtagacttgaacaagtacaaaataccttagcaaaaaggmtgtcaaacagtgaacagaaatatttatcattcttattaaataagaaaatatacctctttt

SEQ ID NO: 83 - DNA, 121 bp, Cucumis melo
agtaaattctgctttttaatggttttcttaggggggaagagggagatgagaactaatgatkacttgcgtgaattcacacaaatctagatacaagtgcatcttacagtttctgtggggcaag

SEQ ID NO: 84 - DNA, 121 bp, Cucumis melo
ccattgagcaacgcagtgagagaattaaaagaaaatctagcgttgtgattaaactcgaagmggagttctctgaccttgttagtcccttaaatatctccagtcctggaaaggagatttcggc

SEQ ID NO: 85 - DNA, 121 bp, Cucumis melo
tcaagatgccgatcttttattctttattgttcgtaatttataccgtgatcttcagtctccragagcactgaggttggaaacagatgatgtcaatgctccccagcggcttccccttttgaaa

SEQ ID NO: 86 - DNA, 121 bp, Cucumis melo
  misc_feature (4)..(4): n is a, c, g, or t
  misc_feature (31)..(31): n is a, c, g, or t
tcgnaaaccgattccacttggggtgtgccanatggctgttcctgattggcttcgagacgtyagccatctcaccaccccgatgctccacagatcagcgagttccaactacctgttgttgtag

SEQ ID NO: 87 - DNA, 121 bp, Cucumis melo
tagcgtaattcgatacttcatataggtagttgtagcgtatttgttatctaccatttgttgwgtggctaagtcaagtttataggaggcttattcacatacatatagattaatgtaccttgtc

SEQ ID NO: 88 - DNA, 121 bp, Cucumis melo
caaaaacctgtgatcgtcaaagaattccgtcaagttttgaatctcgatatactcaagaccygcttctctagccaacctgagtgagttatagccaccatttggataaattcattcagatatt

SEQ ID NO: 89 - DNA, 121 bp, Cucumis melo
ccaagtatgccacaaaccaccgccatatgtctgcacattgaccattagacaattacacttsttcgacgaagacttcggctttaattttaggcatgggctatctgtgtgagcagcaataaca

SEQ ID NO: 90 - DNA, 121 bp, Cucumis melo
  misc_feature (1)..(1): n is a, c, g, or t
  misc_feature (8)..(14): n is a, c, g, or t
  misc_feature (16)..(19): n is a, c, g, or t
  misc_feature (21)..(22): n is a, c, g, or t
  misc_feature (25)..(27): n is a, c, g, or t
  misc_feature (31)..(31): n is a, c, g, or t
  misc_feature (36)..(38): n is a, c, g, or t
naaaaaannnnnnntnnnnannaannncccnttttnnntcatcacctacagtggttcatgrtttcaaaataccttgtttcctgaattataataagctttgttaattaacaaaggtttccac

SEQ ID NO: 91 - DNA, 121 bp, Cucumis melo
catagttctagccgaccttgccaagtcgaccagaactatggtaataaaaattgactagaawatcagacgcataattcaagaacatttcaaaagaatttaagaaactaccttcttgatcctg

SEQ ID NO: 92 - DNA, 121 bp, Cucumis melo
aagaaattatttttcagaatggacatgatgataaataaatgatttaactggattcaggaargagtatttcgagatctcatgggcaggcttgaggtcaatggtggagccatcatttgctgaa

SEQ ID NO: 93 - DNA, 121 bp, Cucumis melo
  misc_feature (4)..(5): n is a, c, g, or t
aganngtagtattgaatttgtgatctacttactgaaggtagaagaattataagttgtccamccatcaacgacgttatggttcccggtgatgatggttcggttaatgccgtctccaataagc

SEQ ID NO: 94 - DNA, 121 bp, Cucumis melo
  misc_feature (95)..(95): n is a, c, g, or t
  misc_feature (106)..(106): n is a, c, g, or t
tcatagttactatacatttggctacaattttcattgtttatagtttcaattcaactatgaraccatactaaaatcgtattgaacaaaacttcaantcttcacgatntagatattactttta

SEQ ID NO: 95 - DNA, 121 bp, Cucumis melo
tcatgtttgttggtaagattgtttgcttcatttttttgatggcttataatttcaggctccwcaaagcagtgctgatgctacagggaattctgatatcgatatccctcctgaattggtgaat

SEQ ID NO: 96 - DNA, 121 bp, Cucumis melo
aaattatgcattctaacaaagaagacttaatcatggcggctgatatggtgtcccttcatcrcactgattatttgtttaccgacggggctccggctccggcagcagtaggcgatagccgact

SEQ ID NO: 97 - DNA, 121 bp, Cucumis melo
attccatgaattgacaagttgaacaatttgggtgtcctgaactcttcttctcttgtgcatyctaagtggtcacattgtgaagaatatttattccctgtttgttggattttgttttagtggt

SEQ ID NO: 98 - DNA, 100 bp, Cucumis melo
ggggacgggagagggggagagaagaattaaggaaggaaayagagagagacatggagatgggagctttgttatatttcggagtttggtgataatggcggag

SEQ ID NO: 99 - DNA, 121 bp, Cucumis melo
ccacaagagggccctgccattaaagtagcttctgagaaaatctttagctttcttgacaatrtgcaggcagagttggaaagtcttaatggtaattctgaaggctttcttcaggtgtgcgaca

SEQ ID NO: 100 - DNA, 121 bp, Cucumis melo
aactcgactttaaattgggtcaacggtgatttaacatgaagttgcagtaagagttgctaasttgaaatctttgcaacaccatctcttattcatcaacctctaaccattaaacacaagaaaa

SEQ ID NO: 101 - DNA, 121 bp, Cucumis melo
  misc_feature (105)..(105): n is a, c, g, or t
caaaatctctgtcagttcaaagtgagtctaaatcgaaactccaccggttttcttctgagcygattcgccttaatgggggacaagctgctggattccattgaaaantattctgccattactt

SEQ ID NO: 102 - DNA, 121 bp, Cucumis melo
  misc_feature (27)..(27): n is a, c, g, or t
attgttgaggggcaaggagtgtttacngtcacgatggtaaggcgagctacatgaaggttcrcctcttgcccgatcagggaagtctgttcctgcactgtcaagactcatccttgaatcagca

SEQ ID NO: 103 - DNA, 121 bp, Cucumis melo
aacgtaacggtgactaaattggacagaaaatgaaccatggagcaaagttaatttcatagcyagggatgctcactggtgtttttgaactgtaatctcgtgaggatattgatgccattttgtt

SEQ ID NO: 104 - DNA, 121 bp, Cucumis melo
caaacatctttgaaactttttcacaccttgaagtcttaaatttgcatgtgccatctgtaaytgaaatgctataaatttcatgtgattatatctgatattttcagtggctggattccttttc

SEQ ID NO: 105 - DNA, 121 bp, Cucumis melo
cttcgagcctctgcggaaatgcttggaaaaggtgggttcggaacttcgtacaaggcgattytggacgacggcaatgtggtggcggtgaaacggctgaaagatgcgcaggttggagggaaac

SEQ ID NO: 106 - DNA, 121 bp, Cucumis melo
ttgagggacttgcaggaattgtgaataaaagccaatcctctagctgctccagcggcgatcytcaacctcgttgtccaatccaacggcgttcgtccagggcctctgtttcctatcaaacagt

SEQ ID NO: 107 - DNA, 111 bp, Cucumis melo
atgcacagaaatgtatgtggcacaagaaacagtctgttaatccttccaattttagaacacraacttccaataatttaccatcagttttcattgaaatattcagatatgcat

SEQ ID NO: 108 - DNA, 121 bp, Cucumis melo
ggcttgtgttctcttctagttaaactgaagatgaactaatgtagaatgtcaaaggtttgcygtaggtgacgtatatgttgtgaagtaaaatttgtttttaaacgtaagtgttgttcagtga

SEQ ID NO: 109 - DNA, 121 bp, Cucumis melo
aagaaagtgggaataaaataaagtaccgatcagaaaagtgctagaaattaagaaatgttawagcaagatagagctcattagtagtggtcgactccactgattaaagagttccgtagaaaaa

SEQ ID NO: 110 - DNA, 91 bp, Cucumis melo
cctgagaattcacccccaccgccaccatcarcacctccagaaacctcacctccctccccagcatcaatacctcctagaaattcaccgccac